European Patent Application EP 4 148 068 A1, published March 15, 2023. Title: ANTI-TIGIT ANTIBODY AND PREPARATION METHOD AND APPLICATION THEREOF. Applicant: HUABO BIOPHARM (SHANGHAI) CO.,LTD. SHANGHAI HUAOTA BIOPHARMACEUTICAL CO., LTD. The sequence listing filed with the application follows.

SEQUENCE LISTING (73 sequences)

SEQ ID NO: 1 - protein, 121 aa, Artificial Sequence
  900424 VH
DVQLQESGPGLVKPSQSLSLTCTVTGYSITSDYAWIWIRQFPGNKVEWMGYITSSGSTSYNPSLKSRISFTRDTSKNQFFLQLTSVTTEDTATYYCARLDFGNYGGAMDYWGQGTSVTVSS

SEQ ID NO: 2 - protein, 107 aa, Artificial Sequence
  900424 VL
DIVMTQSHKFMSTSIGDRVSITCKASQHVSTAVAWYQQKPGQSPKLLIYSASYRYTGVPDRFTGSRSGTDFTFTISSVQAEDLAVYYCQQHYITPYTFGGGTKLEIK

SEQ ID NO: 3 - protein, 9 aa, Artificial Sequence
  HCDR1
GYSITSDYA

SEQ ID NO: 4 - protein, 7 aa, Artificial Sequence
  HCDR2
ITSSGST

SEQ ID NO: 5 - protein, 14 aa, Artificial Sequence
  HCDR3
ARLDFGNYGGAMDY

SEQ ID NO: 6 - protein, 6 aa, Artificial Sequence
  LCDR1
QHVSTA

SEQ ID NO: 7 - protein, 3 aa, Artificial Sequence
  LCDR2
SAS

SEQ ID NO: 8 - protein, 9 aa, Artificial Sequence
  LCDR3
QQHYITPYT

SEQ ID NO: 9 - protein, 121 aa, Artificial Sequence
  HB0030 and HB0031 VH
QVQLQESGPGLVKPSETLSLTCTVSGYSITSDYAWIWIRQPPGKGLEWIGYITSSGSTYYNPSLKSRVTFSVDTSKNQFSLKLSSVTAADTATYYCARLDFGNYGGAMDYWGQGTLVTVSS

SEQ ID NO: 10 - protein, 107 aa, Artificial Sequence
  HB0030 VL
DIQMTQSPSSLSASVGDRVTITCRASQHVSTAVNWYQQKPGKAPKLLIYSASYLYSGVPSRFSGSRSGTDFTLTISSLQPEDFATYYCQQHYITPYTFGQGTKLEIK

SEQ ID NO: 11 - protein, 107 aa, Artificial Sequence
  HB0031 and HB0033 VL
DIQMTQSPSSLSASVGDRVTITCKASQHVSTALAWYQQKPGKAPKLLIYSASYLQSGVPSRFSGSRSGTDFTLTISSLQPEDFATYYCQQHYITPYTFGQGTKLEIK

SEQ ID NO: 12 - protein, 121 aa, Artificial Sequence
  HB0032 VH
QVQLQESGPGLVKPSETLSLTCTVSGYSITSDYAWIWIRQPPGKKLEWIGYITSSGSTYYNPSLKSRVTFSVDTSKNQFSLKLSSVTAADTATYYCARLDFGNYGGAMDYWGQGTLVTVSS

SEQ ID NO: 13 - protein, 107 aa, Artificial Sequence
  HB0032 VL
DIQMTQSPSSLSASVGDRVTITCKASQHVSTAVNWYQQKPGKAPKLLIYSASYRQSGVPSRFSGSGSGTDFTLTISSLQPEDFATYYCQQHYITPYTFGQGTKLEIK

SEQ ID NO: 14 - protein, 121 aa, Artificial Sequence
  HB0033 VH
QVQLQESGPGLVKPSETLSLTCTVSGYSITSDYAWIWIRQPPGNKLEWIGYITSSGSTYYNPSLKSRVTFSVDTSKNQFSLKLSSVTAADTATYYCARLDFGNYGGAMDYWGQGTLVTVSS

SEQ ID NO: 15 - protein, 26 aa, Artificial Sequence [sequence omitted]

SEQ ID NO: 16 - protein, 26 aa, Artificial Sequence [sequence omitted]

SEQ ID NO: 17 - protein, 17 aa, Artificial Sequence
  HB0030 and HB0032 L-FR2
VNWYQQKPGKAPKLLIY

SEQ ID NO: 18 - protein, 17 aa, Artificial Sequence
  HB0031 and HB0033 L-FR2
LAWYQQKPGKAPKLLIY

SEQ ID NO: 19 - protein, 36 aa, Artificial Sequence
  HB0030 L-FR3
YLYSGVPSRFSGSRSGTDFTLTISSLQPEDFATYYC

SEQ ID NO: 20 - protein, 36 aa, Artificial Sequence
  HB0031 and HB0033 L-FR3
YLQSGVPSRFSGSRSGTDFTLTISSLQPEDFATYYC

SEQ ID NO: 21 - protein, 36 aa, Artificial Sequence
  HB0032 L-FR3
YRQSGVPSRFSGSGSGTDFTLTISSLQPEDFATYYC

SEQ ID NO: 22 - protein, 10 aa, Artificial Sequence
  HB0030, HB0031, HB0032 and HB0033 L-FR4
FGQGTKLEIK

SEQ ID NO: 23 - protein, 25 aa, Artificial Sequence
  HB0030, HB0031, HB0032 and HB0033 H-FR1
QVQLQESGPGLVKPSETLSLTCTVS

SEQ ID NO: 24 - protein, 17 aa, Artificial Sequence
  HB0030 and HB0031 H-FR2
WIWIRQPPGKGLEWIGY

SEQ ID NO: 25 - protein, 17 aa, Artificial Sequence
  HB0032 H-FR2
WIWIRQPPGKKLEWIGY

SEQ ID NO: 26 - protein, 17 aa, Artificial Sequence
  HB0033 H-FR2
WIWIRQPPGNKLEWIGY

SEQ ID NO: 27 - protein, 38 aa, Artificial Sequence
  HB0030, HB0031, HB0032 and HB0033 H-FR3
YYNPSLKSRVTFSVDTSKNQFSLKLSSVTAADTATYYC

SEQ ID NO: 28 - protein, 11 aa, Artificial Sequence
  HB0030, HB0031, HB0032 and HB0033 H-FR4
WGQGTLVTVSS

SEQ ID NO: 29 - protein, 329 aa, Artificial Sequence
  human IgG1 constant region wild type
ASTKGPSVFPLAPSSKSTSGGTAALGCLVKDYFPEPVTVSWNSGALTSGVHTFPAVLQSSGLYSLSSVVTVPSSSLGTQTYICNVNHKPSNTKVDKRVEPKSCDKTHTCPPCPAPELLGGPSVFLFPPKPKDTLMISRTPEVTCVVVDVSHEDPEVKFNWYVDGVEVHNAKTKPREEQYNSTYRVVSVLTVLHQDWLNGKEYKCKVSNKALPAPIEKTISKAKGQPREPQVYTLPPSREEMTKNQVSLTCLVKGFYPSDIAVEWESNGQPENNYKTTPPVLDSDGSFFLYSKLTVDKSRWQQGNVFSCSVMHEALHNHYTQKSLSLSPG

SEQ ID NO: 30 - protein, 329 aa, Artificial Sequence
  human IgG1 constant region mutant
ASTKGPSVFPLAPSSKSTSGGTAALGCLVKDYFPEPVTVSWNSGALTSGVHTFPAVLQSSGLYSLSSVVTVPSSSLGTQTYICNVNHKPSNTKVDKRVEPKSCDKTHTCPPCPAPEAAGGPSVFLFPPKPKDTLMISRTPEVTCVVVDVSHEDPEVKFNWYVDGVEVHNAKTKPREEQYNSTYRVVSVLTVLHQDWLNGKEYKCKVSNKALPAPIEKTISKAKGQPREPQVYTLPPSREEMTKNQVSLTCLVKGFYPSDIAVEWESNGQPENNYKTTPPVLDSDGSFFLYSKLTVDKSRWQQGNVFSCSVMHEALHNHYTQKSLSLSPG

SEQ ID NO: 31 - protein, 107 aa, Artificial Sequence [sequence omitted]

SEQ ID NO: 32 - protein, 119 aa, Artificial Sequence
  900423 and 900428VH
DVQLQESGPGLVKPSQSLSLTCTVTGYSITSDYAWNWIRQFPGNRLEWMGYISYSGAPRYNPSLKSRISITRDTSKNQFFLQLSFVTTEDTATYYCASLGTDYYAMDYWGQGTSVIVSS

SEQ ID NO: 33 - protein, 107 aa, Artificial Sequence
  900428VL
DIVMTQSHKFMFTSVGDRVSITCKASQHVSNAVAWYQQKPGQSPKLLIHSASYRYTGVPDRFTGRGSGTDFTFTINSVQAEDLAVYYCQQYYSLPWTFGGGTKLEIK

SEQ ID NO: 34 - protein, 107 aa, Artificial Sequence
  900423VL
DIVMTQSHKFMFTSVGDRVSITCKASQHVSNAVAWYQQKPGQSPKLLIHSASYRYTGVPDRFIGRGSGTDFTFTISSVQAEDLAVYYCQQYYSLPWTFGGGTKLEIK

SEQ ID NO: 35 - protein, 25 aa, Artificial Sequence
  900423, 900424 and 900428 H-FR1
DVQLQESGPGLVKPSQSLSLTCTVT

SEQ ID NO: 36 - protein, 17 aa, Artificial Sequence
  900424 H-FR2
WIWIRQFPGNKVEWMGY

SEQ ID NO: 37 - protein, 17 aa, Artificial Sequence
  900423 and 900428 H-FR2
WNWIRQFPGNRLEWMGY

SEQ ID NO: 38 - protein, 38 aa, Artificial Sequence
  900424 H-FR3
SYNPSLKSRISFTRDTSKNQFFLQLTSVTTEDTATYYC

SEQ ID NO: 39 - protein, 38 aa, Artificial Sequence
  900423 and 900428 H-FR3
RYNPSLKSRISITRDTSKNQFFLQLSFVTTEDTATYYC

SEQ ID NO: 40 - protein, 11 aa, Artificial Sequence
  900424 H-FR4
WGQGTSVTVSS

SEQ ID NO: 41 - protein, 11 aa, Artificial Sequence
  900423 and 900428 H-FR4
WGQGTSVIVSS

SEQ ID NO: 42 - protein, 7 aa, Artificial Sequence
  900423 and 900428 HCDR2
ISYSGAP

SEQ ID NO: 43 - protein, 12 aa, Artificial Sequence
  900423 and 900428 HCDR3
ASLGTDYYAMDY

SEQ ID NO: 44 - protein, 26 aa, Artificial Sequence
  900424 L-FR1
DIVMTQSHKFMSTSIGDRVSITCKAS

SEQ ID NO: 45 - protein, 26 aa, Artificial Sequence
  900423 and 900428 L-FR1
DIVMTQSHKFMFTSVGDRVSITCKAS

SEQ ID NO: 46 - protein, 17 aa, Artificial Sequence
  900424 L-FR2
VAWYQQKPGQSPKLLIY

SEQ ID NO: 47 - protein, 17 aa, Artificial Sequence
  900423 and 900428 L-FR2
VAWYQQKPGQSPKLLIH

SEQ ID NO: 48 - protein, 36 aa, Artificial Sequence
  900428 L-FR3
YRYTGVPDRFTGRGSGTDFTFTINSVQAEDLAVYYC

SEQ ID NO: 49 - protein, 36 aa, Artificial Sequence
  900424 L-FR3
YRYTGVPDRFTGSRSGTDFTFTISSVQAEDLAVYYC

SEQ ID NO: 50 - protein, 36 aa, Artificial Sequence
  900423 L-FR3
YRYTGVPDRFIGRGSGTDFTFTISSVQAEDLAVYYC

SEQ ID NO: 51 - protein, 10 aa, Artificial Sequence
  900423, 900424 and 900428 L-FR4
FGGGTKLEIK

SEQ ID NO: 52 - protein, 6 aa, Artificial Sequence
  900423 and 900428 LCDR1
QHVSNA

SEQ ID NO: 53 - protein, 9 aa, Artificial Sequence
  900423 and 900428 LCDR3
QQYYSLPWT

SEQ ID NO: 54 - protein, 121 aa, Artificial Sequence
  HB0030 and HB0031 VH; HB0032 VH; HB0033 VH
  misc_feature (44)..(44): Xaa = Lys or Asn
  misc_feature (45)..(45): Xaa = Gly or Lys
QVQLQESGPGLVKPSETLSLTCTVSGYSITSDYAWIWIRQPPGXXLEWIGYITSSGSTYYNPSLKSRVTFSVDTSKNQFSLKLSSVTAADTATYYCARLDFGNYGGAMDYWGQGTLVTVSS

SEQ ID NO: 55 - protein, 121 aa, Artificial Sequence
  900424 VH; HB0030 and HB0031 VH; HB0032 VH; HB0033 VH; 900423 and 900428VH
  misc_feature (1)..(1): Xaa = Asp or Gln
  misc_feature (16)..(16): Xaa = Glu or Gln
  misc_feature (17)..(17): Xaa = Ser or Thr
  misc_feature (25)..(25): Xaa = Ser or Thr
  misc_feature (36)..(36): Xaa = Ile or Asn
  misc_feature (41)..(41): Xaa = Phe or Pro
  misc_feature (44)..(44): Xaa = Lys or Asn
  misc_feature (45)..(45): Xaa = Gly, Lys or Arg
  misc_feature (46)..(46): Xaa = Leu or Val
  misc_feature (49)..(49): Xaa = Ile or Met
  misc_feature (53)..(53): Xaa = Ser or Thr
  misc_feature (54)..(54): Xaa = Ser or Tyr
  misc_feature (57)..(57): Xaa = Ala or Ser
  misc_feature (58)..(58): Xaa = Pro or Thr
  misc_feature (59)..(59): Xaa = Arg, Ser or Tyr
  misc_feature (68)..(68): Xaa = Ile or Val
  misc_feature (69)..(69): Xaa = Ser or Thr
  misc_feature (70)..(70): Xaa = Phe or Ile
  misc_feature (71)..(71): Xaa = Ser or Thr
  misc_feature (72)..(72): Xaa = Arg or Val
  misc_feature (80)..(80): Xaa = Phe or Ser
  misc_feature (82)..(82): Xaa = Lys or Gln
  misc_feature (84)..(84): Xaa = Ser or Thr
  misc_feature (85)..(85): Xaa = Phe or Ser
  misc_feature (88)..(88): Xaa = Ala or Thr
  misc_feature (89)..(89): Xaa = Ala or Glu
  misc_feature (98)..(98): Xaa = Arg or Ser
  misc_feature (100)..(100): Xaa = Asp or Gly
  misc_feature (101)..(101): Xaa = Phe or Thr
  misc_feature (102)..(102): Xaa = Asp or Gly
  misc_feature (103)..(103): Xaa = Asn or Tyr
  misc_feature (105)..(105): Xaa = Gly or does not exist
  misc_feature (106)..(106): Xaa = Gly or does not exist
  misc_feature (116)..(116): Xaa = Leu or Ser
  misc_feature (118)..(118): Xaa = Ile or Thr
XVQLQESGPGLVKPSXXLSLTCTVXGYSITSDYAWXWIRQXPGXXXEWXGYIXXSGXXXYNPSLKSRXXXXXDTSKNQFXLXLXXVTXXDTATYYCAXLXXXXYXXAMDYWGQGTXVXVSS

SEQ ID NO: 56 - protein, 7 aa, Artificial Sequence
  900424, HB0030, HB0031, HB0032 and HB0033 HCDR2; 900423 and 900428 HCDR2
  misc_feature (2)..(2): Xaa = Ser or Thr
  misc_feature (3)..(3): Xaa = Ser or Tyr
  misc_feature (6)..(6): Xaa = Ala or Ser
  misc_feature (7)..(7): Xaa = Pro or Thr
IXXSGXX

SEQ ID NO: 57 - protein, 14 aa, Artificial Sequence
  900423 and 900428 HCDR3; 900424, HB0030, HB0031, HB0032 and HB0033 HCDR3
  misc_feature (2)..(2): Xaa = Arg or Ser
  misc_feature (4)..(4): Xaa = Asp or Gly
  misc_feature (5)..(5): Xaa = Phe or Thr
  misc_feature (6)..(6): Xaa = Asp or Gly
  misc_feature (7)..(7): Xaa = Asn or Tyr
  misc_feature (9)..(9): Xaa = Gly or does not exist
  misc_feature (10)..(10): Xaa = Gly or does not exist
AXLXXXXYXXAMDY

SEQ ID NO: 58 - protein, 25 aa, Artificial Sequence
  HB0030, HB0031, HB0032 and HB0033 H-FR1; 900423, 900424 and 900428 H-FR1
  misc_feature (1)..(1): Xaa = Asp or Gln
  misc_feature (16)..(16): Xaa = Glu or Gln
  misc_feature (17)..(17): Xaa = Ser or Thr
  misc_feature (25)..(25): Xaa = Ser or Thr
XVQLQESGPGLVKPSXXLSLTCTVX

SEQ ID NO: 59 - protein, 17 aa, Artificial Sequence
  HB0030 and HB0031 H-FR2; HB0032 H-FR2; HB0033 H-FR2
  misc_feature (10)..(10): Xaa = Lys or Asn
  misc_feature (11)..(11): Xaa = Gly or Lys
WIWIRQPPGXXLEWIGY

SEQ ID NO: 60 - protein, 17 aa, Artificial Sequence
  HB0030 and HB0031 H-FR2; HB0032 H-FR2; HB0033 H-FR2; 900424 H-FR2; 900423 and 900428 H-FR2
  misc_feature (2)..(2): Xaa = Ile or Asn
  misc_feature (7)..(7): Xaa = Phe or Pro
  misc_feature (10)..(10): Xaa = Lys or Asn
  misc_feature (11)..(11): Xaa = Gly, Lys or Arg
  misc_feature (12)..(12): Xaa = Leu or Val
  misc_feature (15)..(15): Xaa = Ile or Met
WXWIRQXPGXXXEWXGY

SEQ ID NO: 61 - protein, 38 aa, Artificial Sequence
  HB0030, HB0031, HB0032 and HB0033 H-FR3; 900423 and 900428 H-FR3; 900424 H-FR3
  misc_feature (1)..(1): Xaa = Arg, Ser or Tyr
  misc_feature (10)..(10): Xaa = Ile or Val
  misc_feature (11)..(11): Xaa = Ser or Thr
  misc_feature (12)..(12): Xaa = Phe or Ile
  misc_feature (13)..(13): Xaa = Ser or Thr
  misc_feature (14)..(14): Xaa = Arg or Val
  misc_feature (22)..(22): Xaa = Phe or Ser
  misc_feature (24)..(24): Xaa = Lys or Gln
  misc_feature (26)..(26): Xaa = Ser or Thr
  misc_feature (27)..(27): Xaa = Phe or Ser
  misc_feature (30)..(30): Xaa = Ala or Thr
  misc_feature (31)..(31): Xaa = Ala or Glu
XYNPSLKSRXXXXXDTSKNQFXLXLXXVTXXDTATYYC

SEQ ID NO: 62 - protein, 11 aa, Artificial Sequence
  HB0030, HB0031, HB0032 and HB0033 H-FR4; 900424 H-FR4; 900423 and 900428 H-FR4
  misc_feature (6)..(6): Xaa = Leu or Ser
  misc_feature (8)..(8): Xaa = Ile or Thr
WGQGTXVXVSS

SEQ ID NO: 63 - protein, 107 aa, Artificial Sequence
  HB0030 VL; HB0031 and HB0033 VL; HB0032 VL
  misc_feature (24)..(24): Xaa = Lys or Arg
  misc_feature (33)..(33): Xaa = Leu or Val
  misc_feature (34)..(34): Xaa = Ala or Asn
  misc_feature (54)..(54): Xaa = Leu or Arg
  misc_feature (55)..(55): Xaa = Gln or Tyr
  misc_feature (66)..(66): Xaa = Gly or Arg
DIQMTQSPSSLSASVGDRVTITCXASQHVSTAXXWYQQKPGKAPKLLIYSASYXXSGVPSRFSGSXSGTDFTLTISSLQPEDFATYYCQQHYITPYTFGQGTKLEIK

SEQ ID NO: 64 - protein, 107 aa, Artificial Sequence
  900424 VL; HB0030 VL; HB0031 and HB0033 VL; HB0032 VL; 900423VL; 900428VL
  misc_feature (3)..(3): Xaa = Gln or Val
  misc_feature (8)..(8): Xaa = His or Pro
  misc_feature (9)..(9): Xaa = Lys or Ser
  misc_feature (10)..(10): Xaa = Phe or Ser
  misc_feature (11)..(11): Xaa = Leu or Met
  misc_feature (12)..(12): Xaa = Phe or Ser
  misc_feature (13)..(13): Xaa = Ala or Thr
  misc_feature (15)..(15): Xaa = Ile or Val
  misc_feature (20)..(20): Xaa = Ser or Thr
  misc_feature (24)..(24): Xaa = Lys or Arg
  misc_feature (31)..(31): Xaa = Asn or Thr
  misc_feature (33)..(33): Xaa = Leu or Val
  misc_feature (34)..(34): Xaa = Ala or Asn
  misc_feature (42)..(42): Xaa = Lys or Gln
  misc_feature (43)..(43): Xaa = Ala or Ser
  misc_feature (49)..(49): Xaa = His or Tyr
  misc_feature (54)..(54): Xaa = Leu or Arg
  misc_feature (55)..(55): Xaa = Gln or Tyr
  misc_feature (56)..(56): Xaa = Ser or Thr
  misc_feature (60)..(60): Xaa = Asp or Ser
  misc_feature (63)..(63): Xaa = Ile, Ser or Thr
  misc_feature (65)..(65): Xaa = Arg or Ser
  misc_feature (66)..(66): Xaa = Gly or Arg
  misc_feature (73)..(73): Xaa = Phe or Leu
  misc_feature (76)..(76): Xaa = Asn or Ser
  misc_feature (78)..(78): Xaa = Leu or Val
  misc_feature (80)..(80): Xaa = Ala or Pro
  misc_feature (83)..(83): Xaa = Phe or Leu
  misc_feature (85)..(85): Xaa = Thr or Val
  misc_feature (91)..(91): Xaa = His or Tyr
  misc_feature (93)..(93): Xaa = Ile or Ser
  misc_feature (94)..(94): Xaa = Leu or Thr
  misc_feature (96)..(96): Xaa = Trp or Tyr
  misc_feature (100)..(100): Xaa = Gly or Gln
DIXMTQSXXXXXXSXGDRVXITCXASQHVSXAXXWYQQKPGXXPKLLIXSASYXXXGVPXRFXGXXSGTDFTXTIXSXQXEDXAXYYCQQXYXXPXTFGXGTKLEIK

SEQ ID NO: 65 - protein, 6 aa, Artificial Sequence
  900424, HB0030, HB0031, HB0032 and HB0033 LCDR1; 900423 and 900428 LCDR1
  misc_feature (5)..(5): Xaa = Asn or Thr
QHVSXA

SEQ ID NO: 66 - protein, 9 aa, Artificial Sequence
  900424, HB0030, HB0031, HB0032 and HB0033 LCDR3; 900423 and 900428 LCDR3
  misc_feature (3)..(3): Xaa = His or Tyr
  misc_feature (5)..(5): Xaa = Ile or Ser
  misc_feature (6)..(6): Xaa = Leu or Thr
  misc_feature (8)..(8): Xaa = Trp or Tyr
QQXYXXPXT

SEQ ID NO: 67 - protein, 26 aa, Artificial Sequence
  HB0031, HB0032 and HB0033 L-FR1; HB0030 L-FR1
  misc_feature (24)..(24): Xaa = Lys or Arg
DIQMTQSPSSLSASVGDRVTITCXAS

SEQ ID NO: 68 - protein, 26 aa, Artificial Sequence
  HB0030 L-FR1; HB0031, HB0032 and HB0033 L-FR1; 900424 L-FR1; 900423 and 900428 L-FR1
  misc_feature (3)..(3): Xaa = Gln or Val
  misc_feature (8)..(8): Xaa = His or Pro
  misc_feature (9)..(9): Xaa = Lys or Ser
  misc_feature (10)..(10): Xaa = Phe or Ser
  misc_feature (11)..(11): Xaa = Leu or Met
  misc_feature (12)..(12): Xaa = Phe or Ser
  misc_feature (13)..(13): Xaa = Ala or Thr
  misc_feature (15)..(15): Xaa = Ile or Val
  misc_feature (20)..(20): Xaa = Ser or Thr
  misc_feature (24)..(24): Xaa = Lys or Arg
DIXMTQSXXXXXXSXGDRVXITCXAS

SEQ ID NO: 69 - protein, 17 aa, Artificial Sequence
  HB0030 and HB0032 L-FR2; HB0031 and HB0033 L-FR2
  misc_feature (1)..(1): Xaa = Leu or Val
  misc_feature (2)..(2): Xaa = Ala or Asn
XXWYQQKPGKAPKLLIY

SEQ ID NO: 70 - protein, 17 aa, Artificial Sequence
  HB0030 and HB0032 L-FR2; HB0031 and HB0033 L-FR2; 900424 L-FR2; 900423 and 900428 L-FR2
  misc_feature (1)..(1): Xaa = Leu or Val
  misc_feature (2)..(2): Xaa = Ala or Asn
  misc_feature (10)..(10): Xaa = Lys or Gln
  misc_feature (11)..(11): Xaa = Ala or Ser
  misc_feature (17)..(17): Xaa = His or Tyr
XXWYQQKPGXXPKLLIX

SEQ ID NO: 71 - protein, 36 aa, Artificial Sequence
  HB0030 L-FR3; HB0031 and HB0033 L-FR3; HB0032 L-FR3
  misc_feature (2)..(2): Xaa = Leu or Arg
  misc_feature (3)..(3): Xaa = Gln or Tyr
  misc_feature (14)..(14): Xaa = Gly or Arg
YXXSGVPSRFSGSXSGTDFTLTISSLQPEDFATYYC

SEQ ID NO: 72 - protein, 36 aa, Artificial Sequence
  HB0030 L-FR3; HB0031 and HB0033 L-FR3; HB0032 L-FR3; 900428 L-FR3; 900424 L-FR3; 900423 L-FR3
  misc_feature (2)..(2): Xaa = Leu or Arg
  misc_feature (3)..(3): Xaa = Gln or Tyr
  misc_feature (4)..(4): Xaa = Ser or Thr
  misc_feature (8)..(8): Xaa = Asp or Ser
  misc_feature (11)..(11): Xaa = Ile, Ser or Thr
  misc_feature (13)..(13): Xaa = Arg or Ser
  misc_feature (14)..(14): Xaa = Gly or Arg
  misc_feature (21)..(21): Xaa = Phe or Leu
  misc_feature (24)..(24): Xaa = Asn or Ser
  misc_feature (26)..(26): Xaa = Leu or Val
  misc_feature (28)..(28): Xaa = Ala or Pro
  misc_feature (31)..(31): Xaa = Phe or Leu
  misc_feature (33)..(33): Xaa = Thr or Val
YXXXGVPXRFXGXXSGTDFTXTIXSXQXEDXAXYYC

SEQ ID NO: 73 - protein, 10 aa, Artificial Sequence
  900423, 900424 and 900428 L-FR4; HB0030, HB0031, HB0032 and HB0033 L-FR4
  misc_feature (3)..(3): Xaa = Gly or Gln
FGXGTKLEIK